European Patent Specification EP 4 003 359 B1, published July 23, 2025. Title: Cobicistat for prevention and/or treatment of coronavirus infections. Applicant: Universität Heidelberg. The sequence listing filed with the application follows.

SEQUENCE LISTING (16 sequences)

SEQ ID NO: 1 - DNA, 19 bp, Artificial Sequence
  Primer
ttaggcctgagttgagtca

SEQ ID NO: 2 - DNA, 20 bp, Artificial Sequence
  Primer
gaccccaaaatcagcgaaat

SEQ ID NO: 3 - DNA, 24 bp, Artificial Sequence
  Primer
tctggttactgccagttgaatctg

SEQ ID NO: 4 - DNA, 20 bp, Artificial Sequence
  Primer
ttacaaacattggccgcaaa

SEQ ID NO: 5 - DNA, 18 bp, Artificial Sequence
  Primer
gcgcgacattccgaagaa

SEQ ID NO: 6 - DNA, 20 bp, Artificial Sequence
  Primer
tgatggctctcatcccagac

SEQ ID NO: 7 - DNA, 20 bp, Artificial Sequence
  Primer
agccccacacttttccatac

SEQ ID NO: 8 - DNA, 20 bp, Artificial Sequence
  Primer
tgatggacctcatcccagac

SEQ ID NO: 9 - DNA, 20 bp, Artificial Sequence
  Primer
cgacaaacaaaagcaccgac

SEQ ID NO: 10 - DNA, 19 bp, Artificial Sequence
  Primer
ttattgactgggctgcgag

SEQ ID NO: 11 - DNA, 20 bp, Artificial Sequence
  Primer
cgacaaacaaaagcaccgag

SEQ ID NO: 12 - DNA, 19 bp, Artificial Sequence
  Primer
taattgattgggccacgag

SEQ ID NO: 13 - DNA, 20 bp, Artificial Sequence
  Primer
cccatcattgcaatagcagg

SEQ ID NO: 14 - DNA, 21 bp, Artificial Sequence
  Primer
tgttcaaacttctgctcctga

SEQ ID NO: 15 - DNA, 21 bp, Artificial Sequence
  Primer
ccactcacagactctcacaac

SEQ ID NO: 16 - DNA, 21 bp, Artificial Sequence
  Primer
ctgcggtacaatcccagaact